European Patent Application EP 4 155 322 A1, published March 29, 2023. Title: ANTI-TRKA ANTIBODY OR ANTIGEN-BINDING FRAGMENT THEREOF, PREPARATION METHOD THEREOF, AND APPLICATION THEREOF. Applicant: XIYUAN ANJIAN MEDCINE (SHANGHAI) CO., LTD. The sequence listing filed with the application follows.

SEQUENCE LISTING (102 sequences)

SEQ ID NO: 1 - protein, 10 aa, Artificial Sequence
GYTFSRYWIE

SEQ ID NO: 2 - protein, 17 aa, Artificial Sequence
EILPGRGVTNYNENFKG

SEQ ID NO: 3 - protein, 10 aa, Artificial Sequence
ARSNYGDYDF

SEQ ID NO: 4 - protein, 10 aa, Artificial Sequence
GYTFTSYWMH

SEQ ID NO: 5 - protein, 17 aa, Artificial Sequence
EINPNNGLTNYDEKFKT

SEQ ID NO: 6 - protein, 11 aa, Artificial Sequence
AKYGNYVAFAF

SEQ ID NO: 7 - protein, 10 aa, Artificial Sequence
GYTFTNYWMH

SEQ ID NO: 8 - protein, 17 aa, Artificial Sequence
EIYPSNGRTNYNEKFKN

SEQ ID NO: 9 - protein, 10 aa, Artificial Sequence
ARSRYDPMED

SEQ ID NO: 10 - protein, 10 aa, Artificial Sequence
GYTFTSYWIH

SEQ ID NO: 11 - protein, 17 aa, Artificial Sequence
EINPNNGLTNYIEKFKN

SEQ ID NO: 12 - protein, 11 aa, Artificial Sequence
AKYGNYVAFAY

SEQ ID NO: 13 - protein, 10 aa, Artificial Sequence
GYTFSRYWIE

SEQ ID NO: 14 - protein, 17 aa, Artificial Sequence
EILPGRSSTNYNEKFKG

SEQ ID NO: 15 - protein, 12 aa, Artificial Sequence
TRVSQLHIYFDY

SEQ ID NO: 16 - protein, 10 aa, Artificial Sequence
GYTFTNYWMH

SEQ ID NO: 17 - protein, 17 aa, Artificial Sequence
EIYPNNGRVNYNEKFKN

SEQ ID NO: 18 - protein, 10 aa, Artificial Sequence
ARSRYDPMED

SEQ ID NO: 19 - protein, 10 aa, Artificial Sequence
GYTFTSYWMH

SEQ ID NO: 20 - protein, 17 aa, Artificial Sequence
EIYSSNGLTNYNEKFKN

SEQ ID NO: 21 - protein, 10 aa, Artificial Sequence
ARHWYVFLDH

SEQ ID NO: 22 - protein, 10 aa, Artificial Sequence
GYTFTNYWMH

SEQ ID NO: 23 - protein, 17 aa, Artificial Sequence
EIYPSNGRTNYNEKFKT

SEQ ID NO: 24 - protein, 10 aa, Artificial Sequence
AGSRYDAMDF

SEQ ID NO: 25 - protein, 14 aa, Artificial Sequence
RSSSGAVTTSNHAN

SEQ ID NO: 26 - protein, 7 aa, Artificial Sequence
GTNNRAP

SEQ ID NO: 27 - protein, 9 aa, Artificial Sequence
ALWYSNHWV

SEQ ID NO: 28 - protein, 11 aa, Artificial Sequence
RASENIYSYVA

SEQ ID NO: 29 - protein, 7 aa, Artificial Sequence
NAKTLAE

SEQ ID NO: 30 - protein, 9 aa, Artificial Sequence
QHHYGIPLT

SEQ ID NO: 31 - protein, 10 aa, Artificial Sequence
SASSSVGYMH

SEQ ID NO: 32 - protein, 7 aa, Artificial Sequence
DTSKLAS

SEQ ID NO: 33 - protein, 9 aa, Artificial Sequence
QQWSSIPLT

SEQ ID NO: 34 - protein, 11 aa, Artificial Sequence
RASENIYTYLA

SEQ ID NO: 35 - protein, 7 aa, Artificial Sequence
NTKTLAE

SEQ ID NO: 36 - protein, 9 aa, Artificial Sequence
QHHYGVPLT

SEQ ID NO: 37 - protein, 16 aa, Artificial Sequence
RSSKSLLHSNGNTYLY

SEQ ID NO: 38 - protein, 7 aa, Artificial Sequence
RMSNLAS

SEQ ID NO: 39 - protein, 9 aa, Artificial Sequence
MQHLEFPLT

SEQ ID NO: 40 - protein, 10 aa, Artificial Sequence
SASSSVGYMH

SEQ ID NO: 41 - protein, 7 aa, Artificial Sequence
DTSKLAS

SEQ ID NO: 42 - protein, 9 aa, Artificial Sequence
QQWSSIPLT

SEQ ID NO: 43 - protein, 14 aa, Artificial Sequence
RSSTGAVTTSNHAN

SEQ ID NO: 44 - protein, 7 aa, Artificial Sequence
GINNRAP

SEQ ID NO: 45 - protein, 9 aa, Artificial Sequence
ALWYSNHWV

SEQ ID NO: 46 - protein, 10 aa, Artificial Sequence
SASSIISYMH

SEQ ID NO: 47 - protein, 7 aa, Artificial Sequence
DTSKLAS

SEQ ID NO: 48 - protein, 9 aa, Artificial Sequence
HQWTSNPLT

SEQ ID NO: 49 - protein, 117 aa, Artificial Sequence
QVQLQQSGAELMKPGASVKISCKAIGYTFSRYWIEWVKQRPGHGLEWIGEILPGRGVTNYNENFKGKATFTVDISSTTTYIQFSSLTSEDSAVYYCARSNYGDYDFWGQGTSLTVSS

SEQ ID NO: 50 - protein, 118 aa, Artificial Sequence
QVQLQQPGAELVKPGASVKLSCKASGYTFTSYWMHWVKQRPGQGLEWIGEINPNNGLTNYDEKFKTKATLTIDKSSRTAYIQLSSLTSEDSAVYYCAKYGNYVAFAFWGQGTLVTVSA

SEQ ID NO: 51 - protein, 117 aa, Artificial Sequence
QVQLQQPGAELVKPGASVKLSCKSSGYTFTNYWMHWVKQRPGQGLEWIGEIYPSNGRTNYNEKFKNRATLTVDISSSTAYMQLSSLTSEDSAVYYCARSRYDPMEDWGQGTSVTVSS

SEQ ID NO: 52 - protein, 118 aa, Artificial Sequence
QVQLQQPGAELVKPGASVQLSCKASGYTFTSYWIHWVKQRPGQGLEWIGEINPNNGLTNYIEKFKNKATLTIDKSSNTAYMQLSGLTPEDSAVYYCAKYGNYVAFAYWGQGTLVTVSA

SEQ ID NO: 53 - protein, 119 aa, Artificial Sequence
QVQLQQSGTELMKPGASVKISCKATGYTFSRYWIEWVKQRPGHGLEWIGEILPGRSSTNYNEKFKGKATFTADTSSNTAYMQLSSLTSEDSAVYYCTRVSQLHIYFDYWGQGTTVTVSS

SEQ ID NO: 54 - protein, 117 aa, Artificial Sequence
QVQLQQPGAELVKPGASVKLSCKSSGYTFTNYWMHWVRQRPGQGLEWIGEIYPNNGRVNYNEKFKNRATLTVDISSSTAYMQLSSLTSEDSAVYYCARSRYDPMEDWGQGTSVTVSS

SEQ ID NO: 55 - protein, 117 aa, Artificial Sequence
QVQLQQPGVELVKPGASVKLSCKTSGYTFTSYWMHWVKQRPGQGLEWIGEIYSSNGLTNYNEKFKNKATLTVDKSSSTAYMQLTSLTSEDSAIYYCARHWYVFLDHWGQGTTLTVSS

SEQ ID NO: 56 - protein, 117 aa, Artificial Sequence
QVQLQQPGAELVKPGASVKLSCKASGYTFTNYWMHWVKQRPGQGLEWIGEIYPSNGRTNYNEKFKTKATLTVDKSSSTAYMHLSSLTSEDSAVYYCAGSRYDAMDFWGQGTSVTVSS

SEQ ID NO: 57 - protein, 109 aa, Artificial Sequence
QTVVTQESALTTSPGETVTLTCRSSSGAVTTSNHANWVQEKPDHLFTSLMGGTNNRAPGVPARFSGSLIGDKAALTITGAQTEDEAIYFCALWYSNHWVFGGGTKLTVL

SEQ ID NO: 58 - protein, 107 aa, Artificial Sequence
DIQMTQSPASLSATVGETVTITCRASENIYSYVAWYQQKQGKSPQLLVHNAKTLAEGVPSRFSGSGSGTQFSLKINGLHPEDFGSYYCQHHYGIPLTFGAGTKLELK

SEQ ID NO: 59 - protein, 106 aa, Artificial Sequence
QIVLTQSPAIMSASPGEKVTMTCSASSSVGYMHWYQQKSGTSPKRWIYDTSKLASGVPTRFSGSGSGTSYSLTISSMEAEDAATYYCQQWSSIPLTFGSGTKLEIK

SEQ ID NO: 60 - protein, 107 aa, Artificial Sequence
DIQMTQSPASLSASVGDTVTITCRASENIYTYLAWYQQKQGKSPQLLVHNTKTLAEGVPSRFSGSGSGTQFSLKISSLQPEDFGTYYCQHHYGVPLTFGAGTKLELK

SEQ ID NO: 61 - protein, 112 aa, Artificial Sequence
DIVMTQVVPSVPVTPGESVSISCRSSKSLLHSNGNTYLYWFQQRPGQSPQLLIYRMSNLASGVPDRFSGSGSGTAFTLRISRVEAEDVAFYYCMQHLEFPLTFGAGTKLELK

SEQ ID NO: 62 - protein, 106 aa, Artificial Sequence
QVVLTQSPAIMSASPGEKVTMTCSASSSVGYMHWYQQKSGTSPKRWIYDTSKLASGVPTRFSGSGSGTSYSLTISSMEAEDAATYFCQQWSSIPLTFGSGTRLEIK

SEQ ID NO: 63 - protein, 109 aa, Artificial Sequence
QAVVTQESALTTSPGETVTLTCRSSTGAVTTSNHANWVQEKPDHLFTGLIGGINNRAPGVPARFSGSLIGDKAALTITGAQTEDEAIYFCALWYSNHWVFGGGTRLTVL

SEQ ID NO: 64 - protein, 106 aa, Artificial Sequence
QIVLTQSPAIMSASPGEKVTMTCSASSIISYMHWYQQKSGTSPKRWIYDTSKLASGVPARFSGSGSGTSYSLTISGMEAEDAATYYCHQWTSNPLTFGGGTKLELK

SEQ ID NO: 65 - DNA, 351 bp, Artificial Sequence
caggttcagctgcagcagtctggagctgagctgatgaagcctggggcctcagtgaagatatcctgcaaggctattgggtacacattcagtaggtactggatagagtgggtaaagcagaggcctggacatggccttgagtggattggagagattttacctggaagaggtgttactaactacaatgagaacttcaagggcaaggccacattcactgtagatatatcctccaccacaacctacattcaattcagcagcctgacatctgaggactctgccgtctattactgtgcaagatcgaattatggtgactacgacttctggggccaaggcacctctctcacagtctcctca

SEQ ID NO: 66 - DNA, 327 bp, Artificial Sequence
cagactgttgtgactcaggaatctgcactcaccacatcacctggtgaaacagtcacactcacttgtcgctcaagttctggggctgttacaactagtaaccatgccaactgggtccaagaaaaacctgatcatttattcactagtctaatgggtggtaccaataaccgagctccaggtgttcctgccagattctcaggctccctgattggcgacaaggctgccctcaccatcacaggggcgcagactgaggatgaggcaatatatttctgtgctctctggtacagcaaccattgggtgttcggtggaggaactaaactgactgtccta

SEQ ID NO: 67 - DNA, 354 bp, Artificial Sequence
caggtccaactgcagcagcctggggctgaactggtgaagcctggggcttcagtgaagctgtcctgcaaggcttccggctacacctttaccagctactggatgcactgggtgaagcagaggcctggacaaggccttgagtggattggagagattaatcctaacaacggtcttactaactacgatgagaaattcaagaccaaggccacactgaccatagacaaatcctccagaacagcctacatacaactcagcagcctgacatctgaggactctgcggtctattactgtgcaaaatatggtaactacgtcgcgtttgctttctggggccaagggactctggtcactgtctctgca

SEQ ID NO: 68 - DNA, 321 bp, Artificial Sequence
gacattcagatgactcagtctccagcctccctatctgcaactgtgggagaaactgtcaccatcacatgtcgagcaagtgaaaatatttacagttatgtagcatggtatcagcagaaacagggaaaatctcctcaactcctggtccataatgcaaaaaccttagcagaaggtgtaccatcaaggttcagtggcagtggatcaggcacacagttttctctgaagatcaacggcctgcaccctgaagattttgggagttattactgtcaacatcattatggtattccgctcacgttcggcgctgggaccaagctggagctgaaa

SEQ ID NO: 69 - DNA, 351 bp, Artificial Sequence
caggtccaactgcagcagcctggggctgaactggtgaagcctggggcttctgtgaagctgtcctgcaagtcttctggctataccttcaccaactactggatgcactgggtgaagcagcggcctggacaaggccttgagtggattggagagatttatcctagcaacggtcgtactaactacaatgagaagttcaaaaacagggccacactgactgtagacatttcctccagcacagcctacatgcaactcagcagcctgacatctgaggactctgcggtctattactgtgcaaggagtaggtacgaccctatggaagactggggtcaaggaacctcagtcaccgtctcctct

SEQ ID NO: 70 - DNA, 318 bp, Artificial Sequence
caaattgttctcacccagtctccagcaatcatgtctgcatctccaggggagaaggtcaccatgacctgcagtgccagctcaagtgtgggttacatgcactggtaccagcagaagtcaggcacctcccccaaaagatggatttatgacacatccaaactggcttctggagtcccaactcgcttcagtggcagtgggtctgggacctcttactctctcacaatcagcagcatggaggctgaggatgctgccacttattactgccagcagtggagtagtatcccactcacgttcggctcggggacaaagttggaaataaag

SEQ ID NO: 71 - DNA, 354 bp, Artificial Sequence
caggtccaactgcagcagcctggggctgaactggtgaagcctggggcttcagtgcagctgtcctgcaaggcttctggctacaccttcaccagttactggatacactgggtgaaacagaggcctggacaaggccttgagtggattggagagattaatcctaacaacggtcttactaactacattgagaaattcaagaacaaggccacactgactattgacaaatcctccaacacagcctacatgcaactcagcggcctgacacctgaggactctgcggtctattactgtgcaaaatatggtaactacgtcgcgtttgcttactggggccaggggactctggtcactgtctctgca

SEQ ID NO: 72 - DNA, 321 bp, Artificial Sequence
gacatccagatgactcagtctccagcctccctatctgcatctgtgggagacactgtcaccatcacatgtcgagcaagtgaaaatatctacacttatttagcttggtatcagcagaaacagggaaaatctcctcaactcctggtccataatacaaaaaccttagcagaaggtgtgccctcaaggttcagtggcagtggatcaggcacacagttttctctgaagatcagcagcctgcagcctgaagattttgggacttattactgtcaacatcattatggtgttccgctcacgttcggtgctgggaccaagctggagctgaaa

SEQ ID NO: 73 - DNA, 357 bp, Artificial Sequence
caggttcagctgcagcagtctggaactgaactgatgaagcctggggcctcagtgaagatatcctgcaaggctactggctacacattcagtagatactggatagagtgggtaaaacagaggcctggacatggccttgagtggattggagagattttacctggaaggagtagtactaactacaatgagaagttcaagggcaaggccacattcactgccgatacatcctccaacacagcctacatgcaactcagcagcctgacatctgaggactctgccgtctattactgtacaagagtttcccaactgcacatttactttgactactggggccaagggaccactgtcacagtctcctcc

SEQ ID NO: 74 - DNA, 336 bp, Artificial Sequence
gatattgtgatgactcaggttgtaccctctgtacctgtcactcctggagagtcagtatccatctcctgcaggtctagtaagagtctcctgcatagtaatggcaacacttacttatattggttccagcagaggccaggccagtctcctcagctcctgatatatcggatgtccaaccttgcctcaggagtcccagacaggttcagtggcagtgggtcaggaactgctttcacattgagaatcagtagagtggaggctgaggatgtggctttttattactgtatgcaacatctagaatttccgctcacgttcggtgctgggaccaagttggagctgaaa

SEQ ID NO: 75 - DNA, 351 bp, Artificial Sequence
caggtccaactgcagcagcctggggctgaactggtgaaacctggggcttcagtgaagctgtcctgcaagtcttctggctataccttcaccaactactggatgcactgggtgaggcagaggcctggacaaggccttgagtggattggagagatctatcctaacaacggtcgtgttaactacaatgagaagttcaagaacagggccacactgactgtagacatatcctccagcacagcctacatgcaactcagcagcctgacatctgaggactctgcggtctattactgtgcaaggagtaggtacgaccctatggaagactggggtcaaggaacctcagtcaccgtctcctct

SEQ ID NO: 76 - DNA, 318 bp, Artificial Sequence
caagttgttctcacccagtctccagcaatcatgtctgcatctccaggggagaaggtcaccatgacctgcagtgccagctcaagtgtaggttacatgcactggtaccagcagaagtcaggcacctcccccaaaagatggatttatgacacatccaaactggcttctggagtcccaactcgcttcagtggcagtgggtctgggacctcttactctctcacaatcagcagcatggaggctgaggatgctgccacttatttctgccagcagtggagtagtatcccactcacgttcggctcggggacaaggttggaaataaag

SEQ ID NO: 77 - DNA, 351 bp, Artificial Sequence
caggtccaactgcagcagcctggggttgaactggtgaagcctggggcttcagtgaagctgtcctgcaagacttctggctacaccttcaccagctactggatgcactgggtgaagcagaggcctggacaaggccttgaatggattggagagatttattccagtaacggtcttactaactacaatgagaagttcaagaataaggccacactgactgtagataaatcctccagcacagcctacatgcaactcaccagcctgacatctgaagactctgcgatctattactgtgcaagacattggtacgtcttccttgaccactggggccaaggcaccactctcacagtctcctca

SEQ ID NO: 78 - DNA, 327 bp, Artificial Sequence
caggctgttgtgactcaggaatctgcactcaccacatcacctggtgaaacagtcacactcacttgtcgctcaagtactggggctgttacaactagtaaccatgccaactgggtccaagaaaaaccagatcatttattcactggtctaataggtggtatcaacaaccgagctccaggtgttcctgccagattctcaggctccctgattggagacaaggctgccctcaccatcacaggggcacagactgaggatgaggcaatatatttctgtgctctatggtacagcaatcattgggtgttcggtggaggaaccagactgactgtccta

SEQ ID NO: 79 - DNA, 351 bp, Artificial Sequence
caggtccaactgcagcagcctggggctgaacttgtgaagcctggggcttcagtgaagctgtcctgtaaggcttctggctacaccttcaccaactactggatgcattgggtgaaacagaggcctggacaaggccttgagtggattggagagatttatcctagcaacggtcgtactaactacaatgagaagttcaagaccaaggccacactgactgtagacaaatcctccagcacagcctacatgcatctcagcagcctgacatctgaggactctgcggtctattactgtgcaggatcgagatacgatgctatggacttctggggtcaaggaacctcagtcaccgtctcctca

SEQ ID NO: 80 - DNA, 318 bp, Artificial Sequence
caaattgttctcacccagtctccagcaatcatgtctgcatctccaggggagaaggtcaccatgacctgcagtgccagctcaattataagttacatgcactggtaccagcagaagtcaggcacctcccccaaaagatggatttatgacacttccaaactggcttctggagtccctgctcgcttcagtggcagtgggtctgggacctcttactctctcacaatcagtggcatggaggctgaagatgctgccacttattactgccaccagtggactagtaacccgctcacgttcggtggtgggaccaagctggaactgaaa

SEQ ID NO: 81 - protein, 117 aa, Artificial Sequence
QVQLVQSGAEVKKPGASVKVSCKSSGYTFTNYWMHWVRQAPGQGLEWMGEIYPNNGRVNYNEKFKNRVTMTVDISISTAYMELSRLRSDDTAVYYCARSRYDPMEDWGQGTTVTVSS

SEQ ID NO: 82 - DNA, 351 bp, Artificial Sequence
caggtgcagctggtgcagagcggagctgaggtgaagaagccaggagcttccgtgaaggtgagctgcaagtccagcggctacaccttcacaaactattggatgcactgggtgaggcaggctccaggacagggactggagtggatgggcgagatctaccctaacaatggcagggtgaactacaacgagaagtttaagaacagagtgaccatgacagtggacatcagcatctctaccgcttacatggagctgtctaggctgcggtccgacgatacagccgtgtactattgtgctagatctcgctatgaccccatggaggattggggccagggcaccacagtgaccgtgtcttcc

SEQ ID NO: 83 - protein, 106 aa, Artificial Sequence
DVQLTQSPSSLSASVGDRVTITCSASSSVGYMHWYQQKPGKAPKRLIYDTSKLASGVPSRFSGSGSGTDYTLTISSLQPEDFATYFCQQWSSIPLTFGQGTRLEIK

SEQ ID NO: 84 - DNA, 318 bp, Artificial Sequence
gacgtgcagctgacccagtctccttccagcctgtccgccagcgtgggcgatagagtgaccatcacatgctccgcttcttccagcgtgggctacatgcactggtatcagcagaagcccggcaaggcccctaagaggctgatctacgacacatctaagctggcttccggagtgccaagccggttctctggctccggcagcggaaccgactacaccctgacaatctcttccctgcagccagaggatttcgccacatatttttgtcagcagtggagctctatccccctgacctttggccagggcacacgcctggagatcaag

SEQ ID NO: 85 - protein, 117 aa, Artificial Sequence
QVQLVQSGAEVKKPGASVKVSCKSSGYTFTNYWMHWVRQAPGQGLEWIGEIYPNNGRVNYNEKFKNRATLTVDISISTAYMELSRLRSDDTAVYYCARSRYDPMEDWGQGTTVTVSS

SEQ ID NO: 86 - DNA, 351 bp, Artificial Sequence
caggtgcagctggtgcagagcggagctgaggtgaagaagccaggagcttccgtgaaggtgagctgcaagtccagcggctacaccttcacaaactattggatgcactgggtgaggcaggctccaggacagggactggagtggatcggcgagatctaccctaacaatggcagggtgaactacaacgagaagtttaagaacagagccaccctgacagtggacatcagcatctctaccgcttacatggagctgtctaggctgcggtccgacgatacagccgtgtactattgtgctagatctcgctatgaccccatggaggattggggccagggcaccacagtgaccgtgtcttcc

SEQ ID NO: 87 - protein, 106 aa, Artificial Sequence
DVQLTQSPSSLSASVGDRVTITCSASSSVGYMHWYQQKPGKAPKRWIYDTSKLASGVPSRFSGSGSGTDYTLTISSLQPEDFATYFCQQWSSIPLTFGQGTRLEIK

SEQ ID NO: 88 - DNA, 318 bp, Artificial Sequence
gacgtgcagctgacccagtctccttccagcctgtccgccagcgtgggcgatagagtgaccatcacatgctccgcttcttccagcgtgggctacatgcactggtatcagcagaagcccggcaaggcccctaagaggtggatctacgacacatctaagctggcttccggagtgccaagccggttctctggctccggcagcggaaccgactacaccctgacaatctcttccctgcagccagaggatttcgccacatatttttgtcagcagtggagctctatccccctgacctttggccagggcacacgcctggagatcaag

SEQ ID NO: 89 - protein, 117 aa, Artificial Sequence
QVQLVQSGAEVKKPGSSVKVSCKSSGYTFTNYWMHWVRQAPGQGLEWIGEIYPNNGRVNYNEKFKNRATLTVDISTSTAYMELSSLRSEDTAVYYCARSRYDPMEDWGQGTTVTVSS

SEQ ID NO: 90 - DNA, 351 bp, Artificial Sequence
caggtgcagctggtgcagtccggagctgaggtgaagaagccaggctccagcgtgaaggtgagctgcaagtcttccggctacaccttcacaaactattggatgcactgggtgaggcaggctccaggacagggactggagtggatcggcgagatctaccctaacaatggcagagtgaactacaacgagaagtttaagaaccgcgccaccctgacagtggacatctctacctccacagcttacatggagctgagctctctgagaagcgaggataccgccgtgtactattgtgctaggtctcggtatgaccccatggaggattggggccagggcaccacagtgacagtgtccagc

SEQ ID NO: 91 - protein, 106 aa, Artificial Sequence
QVQLTQSPSSLSASVGDRVTITCSASSSVGYMHWYQQKPGKAPKRLIYDTSKLASGVPSRFSGSGSGTDYTLTISSLQPEDFATYFCQQWSSIPLTFGQGTRLEIK

SEQ ID NO: 92 - DNA, 318 bp, Artificial Sequence
caggtgcagctgacccagtctccttccagcctgtccgccagcgtgggcgacagagtgaccatcacatgctccgcttcttccagcgtgggctacatgcactggtatcagcagaagcccggcaaggcccctaagaggctgatctacgatacatctaagctggcttccggagtgccaagccggttctctggctccggcagcggaaccgactacaccctgacaatctcttccctgcagccagaggatttcgccacatatttttgtcagcagtggagctctatccccctgacctttggccagggcacacgcctggagatcaag

SEQ ID NO: 93 - protein, 106 aa, Artificial Sequence
QVQLTQSPSSLSASVGDRVTITCSASSSVGYMHWYQQKPGKAPKRWIYDTSKLASGVPSRFSGSGSGTDYTLTISSLQPEDFATYFCQQWSSIPLTFGQGTRLEIK

SEQ ID NO: 94 - DNA, 318 bp, Artificial Sequence
caggtgcagctgacccagtctccttccagcctgtccgccagcgtgggcgacagagtgaccatcacatgctccgcttcttccagcgtgggctacatgcactggtatcagcagaagcccggcaaggcccctaagaggtggatctacgatacatctaagctggcttccggagtgccaagccggttctctggctccggcagcggaaccgactacaccctgacaatctcttccctgcagccagaggatttcgccacatatttttgtcagcagtggagctctatccccctgacctttggccagggcacacgcctggagatcaag

SEQ ID NO: 95 - protein, 106 aa, Artificial Sequence
EVVLTQSPATLSLSPGERATLSCSASSSVGYMHWYQQKPGQAPRRWIYDTSKLASGVPARFSGSGSGTDYTLTISSLEPEDAAVYFCQQWSSIPLTFGQGTRLEIK

SEQ ID NO: 96 - DNA, 318 bp, Artificial Sequence
gaggtggtgctgacccagtccccagccacactgagcctgtctccaggagagagagccaccctgtcctgctccgcctccagctctgtgggctacatgcactggtatcagcagaagccaggacaggctcctaggcggtggatctacgacacctctaagctggcttccggagtgccagctcgcttctctggctccggcagcggcacagactacaccctgacaatctccagcctggagcctgaggatgccgccgtgtacttctgtcagcagtggtcttccatcccactgacctttggccagggcacaaggctggagatcaag

SEQ ID NO: 97 - protein, 117 aa, Artificial Sequence
QVQLVQSGAEVKKPGASVKVSCKSSGYTFTNYWMHWVRQAPGQGLEWMGEIYPNSGRVNYNEKFKNRVTMTVDISISTAYMELSRLRSDDTAVYYCARSRYDPMEDWGQGTTVTVSS

SEQ ID NO: 98 - DNA, 351 bp, Artificial Sequence
caggtgcagctggtgcagtccggcgccgaggtgaagaagcccggcgcttctgtgaaggtgagctgcaagagctccggctacacctttaccaattattggatgcactgggtgaggcaggctcccggccagggactggagtggatgggcgagatatatcccaatagcggccgggtgaattataatgagaagtttaagaatcgggtgaccatgaccgtggatatcagcatctccaccgcctacatggagctgagcaggctgaggagcgatgacaccgctgtgtactactgcgctaggtccaggtatgaccccatggaggattggggccagggcaccaccgtgaccgtgagcagc

SEQ ID NO: 99 - protein, 117 aa, Artificial Sequence
QVQLVQSGAEVKKPGASVKVSCKSSGYTFTNYWMHWVRQAPGQGLEWMGEIYPNQGRVNYNEKFKNRVTMTVDISISTAYMELSRLRSDDTAVYYCARSRYDPMEDWGQGTTVTVSS

SEQ ID NO: 100 - DNA, 351 bp, Artificial Sequence
caggtgcagctggtgcagagcggcgccgaggtgaagaagcccggcgcttccgtgaaggtgtcctgtaagtccagcggctataccttcaccaactattggatgcactgggtgaggcaggcccctggccagggactggagtggatgggcgagatatatcctaaccagggccgggtgaattataacgagaagttcaagaatagggtgaccatgaccgtggacatctccatcagcaccgcttacatggagctgtccaggctgcggagcgacgataccgccgtgtactactgtgccaggtcccggtatgatcccatggaggactggggccagggcaccaccgtgaccgtgagcagc

SEQ ID NO: 101 - protein, 117 aa, Artificial Sequence
QVQLVQSGAEVKKPGASVKVSCKSSGYTFTNYWMHWVRQAPGQGLEWMGEIYPNNARVNYNEKFKNRVTMTVDISISTAYMELSRLRSDDTAVYYCARSRYDPMEDWGQGTTVTVSS

SEQ ID NO: 102 - DNA, 351 bp, Artificial Sequence
caggtgcagctggtgcagtccggcgccgaggtgaagaagcccggcgcttctgtgaaggtgtcctgtaagagcagcggctacacctttaccaattattggatgcactgggtgaggcaggcccccggccagggattggagtggatgggcgagatatatcctaacaatgccagggtgaactataatgagaagtttaagaaccgggtgaccatgaccgtggacatcagcatctccaccgcctatatggagctgagccggctgcggtccgacgacaccgctgtgtactactgcgcccggtcccggtatgatcctatggaggactggggccagggcaccaccgtgaccgtgagctcc